European Patent Application EP 4 442 256 A1, published October 9, 2024. Title: LIPID NANOPARTICLE COMPOSITIONS. Applicant: Københavns Universitet. Application EP, filed April 4, 2023. The sequence listing filed with the application follows.

SEQUENCE LISTING (11 sequences)

SEQ ID NO: 1 - RNA, 1653 nt, synthetic construct
  source 1..1653: mol_type = other RNA
atggaggacgccaagaacatcaagaagggccccgcccccttctaccccctggaggacggcaccgccggcgagcagctgcacaaggccatgaagcggtacgccctggtgcccggcaccatcgccttcaccgacgcccacatcgaggtggacatcacctacgccgagtacttcgagatgagcgtgcggctggccgaggccatgaagcggtacggcctgaacaccaaccaccggatcgtggtgtgcagcgagaacagcctgcagttcttcatgcccgtgctgggcgccctgttcatcggcgtggccgtggcccccgccaacgacatctacaacgagcgggagctgctgaacagcatgggcatcagccagcccaccgtggtgttcgtgagcaagaagggcctgcagaagatcctgaacgtgcagaagaagctgcccatcatccagaagatcatcatcatggacagcaagaccgactaccagggcttccagagcatgtacaccttcgtgaccagccacctgccccccggcttcaacgagtacgacttcgtgcccgagagcttcgaccgggacaagaccatcgccctgatcatgaacagcagcggcagcaccggcctgcccaagggcgtggccctgccccaccggaccgcctgcgtgcggttcagccacgcccgggaccccatcttcggcaaccagatcatccccgacaccgccatcctgagcgtggtgcccttccaccacggcttcggcatgttcaccaccctgggctacctgatctgcggcttccgggtggtgctgatgtaccggttcgaggaggagctgttcctgcggagcctgcaggactacaagatccagagcgccctgctggtgcccaccctgttcagcttcttcgccaagagcaccctgatcgacaagtacgacctgagcaacctgcacgagatcgccagcggcggcgcccccctgagcaaggaggtgggcgaggccgtggccaagcggttccacctgcccggcatccggcagggctacggcctgaccgagaccaccagcgccatcctgatcacccccgagggcgacgacaagcccggcgccgtgggcaaggtggtgcccttcttcgaggccaaggtggtggacctggacaccggcaagaccctgggcgtgaaccagcggggcgagctgtgcgtgcggggccccatgatcatgagcggctacgtgaacaaccccgaggccaccaacgccctgatcgacaaggacggctggctgcacagcggcgacatcgcctactgggacgaggacgagcacttcttcatcgtggaccggctgaagagcctgatcaagtacaagggctaccaggtggcccccgccgagctggagagcatcctgctgcagcaccccaacatcttcgacgccggcgtggccggcctgcccgacgacgacgccggcgagctgcccgccgccgtggtggtgctggagcacggcaagaccatgaccgagaaggagatcgtggactacgtggccagccaggtgaccaccgccaagaagctgcggggcggcgtggtgttcgtggacgaggtgcccaagggcctgaccggcaagctggacgcccggaagatccgggagatcctgatcaaggccaagaagggcggcaagatcgccgtgtga

SEQ ID NO: 2 - RNA, 1161 nt, synthetic construct
  source 1..1161: mol_type = other RNA
atgggcagcatcggcgccgccagcatggagttctgcttcgacgtgttcaaggagctgaaggtgcaccacgccaacgagaacatcttctactgccccatcgccatcatgagcgccctggccatggtgtacctgggcgccaaggacagcacccggacccagatcaacaaggtggtgcggttcgacaagctgcccggcttcggcgacagcatcgaggcccagtgcggcaccagcgtgaacgtgcacagcagcctgcgggacatcctgaaccagatcaccaagcccaacgacgtgtacagcttcagcctggccagccggctgtacgccgaggagcggtaccccatcctgcccgagtacctgcagtgcgtgaaggagctgtaccggggcggcctggagcccatcaacttccagaccgccgccgaccaggcccgggagctgatcaacagctgggtggagagccagaccaacggcatcatccggaacgtgctgcagcccagcagcgtggacagccagaccgccatggtgctggtgaacgccatcgtgttcaagggcctgtgggagaagaccttcaaggacgaggacacccaggccatgcccttccgggtgaccgagcaggagagcaagcccgtgcagatgatgtaccagatcggcctgttccgggtggccagcatggccagcgagaagatgaagatcctggagctgcccttcgccagcggcaccatgagcatgctggtgctgctgcccgacgaggtgagcggcctggagcagctggagagcatcatcaacttcgagaagctgaccgagtggaccagcagcaacgtgatggaggagcggaagatcaaggtgtacctgccccggatgaagatggaggagaagtacaacctgaccagcgtgctgatggccatgggcatcaccgacgtgttcagcagcagcgccaacctgagcggcatcagcagcgccgagagcctgaagatcagccaggccgtgcacgccgcccacgccgagatcaacgaggccggccgggaggtggtgggcagcgccgaggccggcgtggacgccgccagcgtgagcgaggagttccgggccgaccaccccttcctgttctgcatcaagcacatcgccaccaacgccgtgctgttcttcggccggtgcgtgagcccctga

SEQ ID NO: 3 - DNA, 25 bp, synthetic construct
  misc_feature 1..23: note = RNA
  misc_feature 24..25: note = DNA
  source 1..25: mol_type = other DNA
gtctcagcctcttctcattcctgct

SEQ ID NO: 4 - RNA, 27 nt, synthetic construct
  source 1..27: mol_type = other RNA
agcaggaatgagaagaggctgagacat

SEQ ID NO: 5 - RNA, 3822 nt, Severe acute respiratory syndrome-related coronavirus
  source 1..3822: mol_type = mRNA
atgttcgtgttcctggtgctgctgcccctggtgagctctcagtgcgtgaacctgaccacaagaacacagctgccccccgcctacaccaacagcttcacaagaggagtgtactaccccgacaaggtgttcagaagcagcgtgcttcacagcacccaagacctgtttctgcctttctttagtaacgtgacctggttccacgccatccacgtgagcggcaccaacggcaccaagagattcgacaaccccgtgctgcccttcaacgacggcgtgtacttcgctagcaccgagaagagcaacatcatcagaggctggatcttcggcaccaccctagatagcaagacacagagcctgctgatcgtgaacaatgccaccaacgtggtgatcaaggtgtgcgagtttcagttctgcaacgaccccttcctgggcgtgtattaccacaaaaacaacaagagctggatggagagcgagttcagagtgtacagcagcgccaacaactgcaccttcgagtacgtgtctcagcccttcctgatggacctggagggcaagcaaggcaatttcaagaacctgagagagttcgtgttcaagaacatcgacggctacttcaagatctacagcaagcacacccccatcaacctggtgagagacctgccccaaggcttcagcgccctggagcccctggtggacctgcccatcggcatcaacatcacaagatttcagaccctgctggccctgcaccgaagctatctaacacccggggacagcagctccggttggacagcgggcgccgccgcctattacgtgggctacctgcagcctagaaccttcctgctgaagtacaacgagaacggcaccatcaccgacgccgttgactgcgccctggaccccctgagcgagaccaagtgcaccctgaagagcttcaccgtggagaagggcatctatcagacaagcaacttcagagtgcagcccaccgagagcatcgtgagattccccaacatcaccaacctgtgccccttcggcgaggtgttcaacgccacaagattcgctagcgtgtacgcctggaacagaaagagaatcagcaactgcgtggccgactacagcgtgctgtacaacagcgctagcttcagcaccttcaagtgttacggcgtgagccccaccaagctgaacgacctgtgcttcaccaacgtgtacgccgacagcttcgtgatcagaggcgacgaggtgagacagatcgcccccgggcagaccggcaagatcgccgactacaactacaagctgcccgacgacttcaccggctgcgtgatcgcttggaacagcaataacctggatagcaaggtgggaggcaactacaactacctgtacagactgttcagaaagagcaacctgaagcccttcgagagagacatcagcaccgagatctaccaagccggcagcaccccctgcaacggcgtgaagggcttcaactgctacttccccctgcagagctacggctttcagcccacctacggcgtgggctatcagccctacagagtggtggtgctgagcttcgagctgctgcacgcccccgctaccgtgtgcggccccaagaagagcaccaacctggtgaagaacaagtgcgtgaacttcaactttaacggtctgaccggtaccggcgtgctgaccgagagcaacaagaagttcctcccatttcagcagttcggcagagacatcgccgacaccactgacgccgtaagagaccctcagaccctggagatcctggacatcacgccatgcagcttcggaggcgtgagcgtgatcacccccggcaccaacacaagcaaccaagtggccgtgctgtaccaaggcgtgaactgcaccgaggtgcccgtggccatccacgccgatcagctgacccccacctggcgcgtctatagcaccggaagcaacgtgtttcagacaagagccggctgcctgatcggcgccgagcacgtgaacaacagctacgagtgcgacatccccatcggcgccggcatctgcgctagctatcagacacagaccaacagccctagaagagctagaagcgtggcttctcagagcatcatcgcctacaccatgagcctgggcgccgagaacagcgtggcctacagcaacaacagcatcgccatccccaccaacttcaccatcagcgtgaccaccgagattctgcctgtgagcatgaccaagacaagcgtggactgcaccatgtacatctgcggcgacagcaccgagtgcagcaacctgctgctgcagtacggcagcttctgcacacagctgaacagagccctgaccggcatcgccgtggagcaagacaagaacacccaagaggtgttcgcccaagtgaagcagatctacaagaccccccccatcaaggacttcggcggcttcaacttcagccaaatcctgcccgaccctagcaagcctagcaagcggagcttcatcgaggacctgctgttcaacaaggtgaccctggccgacgccggcttcatcaagcagtacggcgactgcctgggcgacatcgcagctagagacctgatctgcgctcagaagttcaatggtctgaccgtgctcccccccctgctgaccgacgagatgatcgctcagtatacctccgccctgttagccggaacgatcacaagcggctggactttcggggccggtgcggccctacagatccccttcgccatgcagatggcctacagattcaacggcatcggcgtgacacagaacgtgctgtacgagaatcagaagctgatcgccaatcagttcaacagcgccatcggcaagatccaagacagcctgagcagcaccgctagcgccctgggcaagctgcaagacgtggtgaatcagaacgcccaagccctgaacaccctggtgaagcagctgagcagcaacttcggcgccatcagcagcgtgctgaatgatatcctgagcagactggacaaggtggaggccgaggtgcagatcgacagactgatcaccggcagactgcagagcctgcagacctacgtgacacagcagctgatcagagccgccgagatcagagctagcgccaacctggccgccaccaagatgagcgagtgcgtgctggggcagagcaagagagtggacttctgcggcaagggctaccacctgatgagcttccctcagagcgccccccacggcgtggtgttcctgcacgtgacctacgtgcccgcccaagagaagaacttcactacggcacctgccatctgccacgacggcaaggcccacttccctagagagggcgtgttcgtgagcaacggcacccactggttcgtgacacagagaaacttctacgagcctcagatcatcaccaccgacaacaccttcgtgagcggcaactgcgacgtggtgatcggtatcgttaataataccgtgtacgaccccctacagcccgaactggacagcttcaaggaggagctggacaagtacttcaaaaaccacactagccccgacgtggacctgggtgatattagcggcatcaacgctagcgtggtgaacattcagaaggagatcgaccggctgaatgaggtggccaagaacctgaacgagagcctgatcgacctgcaagagctgggcaagtacgagcagtacatcaagtggccctggtacatctggctgggcttcatcgccggcctgatcgccatcgtgatggtgaccatcatgctgtgctgcatgacaagctgttgcagctgcctgaaaggttgctgcagctgtggctcgtgctgcaagttcgacgaggacgacagcgagcccgtgctgaagggcgtgaagctgcactacacctga

SEQ ID NO: 6 - protein, 8 aa, synthetic construct
SIINFEKL

SEQ ID NO: 7 - protein, 17 aa, synthetic construct
ISQAVHAAHAEINEAGR

SEQ ID NO: 8 - RNA, 285 nt, Mycobacterium tuberculosis
  source 1..285: mol_type = mRNA
atgaccgaacagcagtggaactttgcgggcattgaagcggcggcgagcgcgattcagggcaacgtgaccagcattcatagcctgctggatgaaggcaaacagagcctgaccaaactggcggcggcgtggggcggcagcggcagcgaagcgtatcagggcgtgcagcagaaatgggatgcgaccgcgaccgaactgaacaacgcgctgcagaacctggcgcgcaccattagcgaagcgggccaggcgatggcgagcaccgaaggcaacgtgaccggcatgtttgcg

SEQ ID NO: 9 - RNA, 975 nt, Mycobacterium tuberculosis
  source 1..975: mol_type = mRNA
atgaccgatgtgagccgcaaaattcgcgcgtggggccgccgcctgatgattggcaccgcggcggcggtggtgctgccgggcctggtgggcctggcgggcggcgcggcgaccgcgggcgcgtttagccgcccgggcctgccggtggaatatctgcaggtgccgagcccgagcatgggccgcgatattaaagtgcagtttcagagcggcggcaacaacagcccggcggtgtatctgctggatggcctgcgcgcgcaggatgattataacggctgggatattaacaccccggcgtttgaatggtattatcagagcggcctgagcattgtgatgccggtgggcggccagagcagcttttatagcgattggtatagcccggcgtgcggcaaagcgggctgccagacctataaatgggaaacctttctgaccagcgaactgccgcagtggctgagcgcgaaccgcgcggtgaaaccgaccggcagcgcggcgattggcctgagcatggcgggcagcagcgcgatgattctggcggcgtatcatccgcagcagtttatttatgcgggcagcctgagcgcgctgctggatccgagccagggcatgggcccgagcctgattggcctggcgatgggcgatgcgggcggctataaagcggcgaacatgtggggcccgagcagcgatccggcgtgggaacgcaacgatccgacccagcagattccgaaactggtggcgaacaacacccgcctgtgggtgtattgcggcaacggcaccccgaacgaactgggcggcgcgaacattccggcggaatttctgaaaaactttgtgcgcagcagcaacctgaaatttcaggatgcgtataacgcggcgggcggccataacgcggtgtttaactttccgccgaacggcacccatagctgggaatattggggcgcgcagctgaacgcgatgaaaggcgatctgcagagcagcctgggcgcgggc

SEQ ID NO: 10 - RNA, 1194 nt, synthetic construct
  source 1..1194: mol_type = other RNA
atgatgagaaaattagctattttatctgtttcttcctttttatttgttgaggccttattccaggaataccagtgctatggaagttcgtcaaacacaagggttctaaatgaattaaattatgataatgcaggcactaatttatataatgaattagaaatgaattattatgggaaacaggaaaattggtatagtcttaaaaaaaatagtagatcacttggagaaaatgatgatggaaataacgaagacaacgagaaattaaggaaaccaaaacataaaaaattaaagcaaccagcggatggtaatcctgatccaaatgcaaacccaaatgtagatcccaatgccaacccaaatgtagatccaaatgcaaacccaaatgtagatccaaatgcaaacccaaatgcaaacccaaatgcaaacccaaatgcaaacccaaatgcaaacccaaatgcaaacccaaatgcaaacccaaatgcaaacccaaatgcaaacccaaatgcaaacccaaatgcaaacccaaatgcaaacccaaatgcaaacccaaatgcaaaccccaatgcaaatcctaatgcaaacccaaatgcaaacccaaacgtagatcctaatgcaaatccaaatgcaaacccaaacgcaaaccccaatgcaaatcctaatgcaaaccccaatgcaaatcctaatgcaaatcctaatgccaatccaaatgcaaatccaaatgcaaacccaaacgcaaaccccaatgcaaatcctaatgccaatccaaatgcaaatccaaatgcaaacccaaatgcaaacccaaatgcaaaccccaatgcaaatcctaataaaaacaatcaaggtaatggacaaggtcacaatatgccaaatgacccaaaccgaaatgtagatgaaaatgctaatgccaacagtgctgtaaaaaataataataacgaagaaccaagtgataagcacataaaagaatatttaaacaaaatacaaaattctctttcaactgaatggtccccatgtagtgtaacttgtggaaatggtattcaagttagaataaagcctggctctgctaataaacctaaagacgaattagattatgcaaatgatattgaaaaaaaaatttgtaaaatggaaaaatgttccagtgtgtttaatgtcgtaaatagttcaataggattaataatggtattatccttcttgttccttaattag

SEQ ID NO: 11 - RNA, 1942 nt, synthetic construct
  source 1..1942: mol_type = other RNA
gggagaaagcttaccatggagctgcccatcctcaaggccaacgccatcaccaccatcctggcggccgtgacgttctgcttcgccagctcccagaacatcaccgaggagttctaccagagcacctgctccgccgtcagcaagggctacctgtccgccctccggaccgggtggtacacgagcgtgatcaccatcgagctgtccaacatcaaggagaacaagtgcaacggcaccgacgcgaaggtgaagctgatcaaccaggagctcgacaagtacaagaacgccgtcaccgagctgcagctgctcatgcagagcacgaccgccgccaacaaccgcgcgcggcgcgagctgccgcggttcatgaactacaccctgaacaacaccaagaagacgaacgtgaccctctccaagaagcgcaagcggcgcttcctggggttcctgctcggcgtggggagcgccatcgcctccggcatcgccgtcagcaaggtgctgcacctggagggcgaggtgaacaagatcaagtccgccctcctgagcaccaacaaggcggtcgtgtccctgagcaacggggtgtccgtcctcaccagcaaggtgctggacctgaagaactacatcgacaagcagctcctgcccatcgtgaacaagcagtcctgccggatcagcaacatcgagacggtcatcgagttccagcagaagaacaaccgcctgctcgagatcacccgggagttcagcgtgaacgccggcgtgaccacccccgtctccacgtacatgctgaccaacagcgagctgctctccctgatcaacgacatgcccatcaccaacgaccagaagaagctgatgagcaacaacgtgcagatcgtgcgccagcagtcctacagcatcatgtccatcatcaaggaggaggtcctcgcctacgtggtgcagctgccgctgtacggggtcatcgacaccccctgctggaagctccacacgagccccctgtgcaccaccaacaccaaggagggctccaacatctgcctgacgcggaccgaccgcgggtggtactgcgacaacgccggcagcgtgtccttcttcccccaggccgagacctgcaaggtccagagcaaccgggtgttctgcgacaccatgaactccctcacgctgccgagcgaggtgaacctgtgcaacgtcgacatcttcaaccccaagtacgactgcaagatcatgacctccaagaccgacgtgagctccagcgtgatcacctccctcggcgcgatcgtcagctgctacgggaagacgaagtgcaccgccagcaacaagaaccgcggcatcatcaagaccttctccaacgggtgcgactacgtgagcaacaagggcgtggacaccgtctccgtgggcaacaccctgtactacgtgaacaagcaggaggggaagagcctgtacgtcaagggcgagcccatcatcaacttctacgaccccctcgtgttcccgtccgacgagttcgacgccagcatctcccaggtgaacgagaagatcaaccagagcctggccttcatccggaagtccgacgagctgctgcaccacgtcaacgccgggaagagcacgaccaacatcatgatcaccaccatcatcatcgtgatcatcgtgatcctcctgtccctgatcgcggtcggcctcctgctgtactgcaaggcccgcagcacgcccgtgaccctctccaaggaccagctgagcgggatcaacaacatcgccttctccaactgaggactagttataagactgactagcccgatgggcctcccaacgggccctcctcccctccttgcaccgagattaataaaaaaaaaaaaaaaaaaaaaaaaaaaaaaaaaaaaaaaaaaaaaaaaaaaaaaaaaaaaaaaatgcatcccccccccccccccccccccccccccccccaaaggctcttttcagagccaccagaatt